European Patent Application EP 4 552 498 A1, published May 14, 2025. Title: METHOD FOR PREVENTING INSECT DAMAGE TO PLANTS. Applicant: Ajinomoto Co., Inc. Application WO PCT/JP2023/024818, filed July 4, 2023. The sequence listing filed with the application follows.

SEQUENCE LISTING (4 sequences)

SEQ ID NO: 1 - DNA, 24 bp, synthetic construct
  misc_feature 1..24: note = primer
  source 1..24: mol_type = other DNA
cgttttacactcaagatccagttg

SEQ ID NO: 2 - DNA, 21 bp, synthetic construct
  misc_feature 1..21: note = primer
  source 1..21: mol_type = other DNA
attatcaaactcagaggcggg

SEQ ID NO: 3 - DNA, 20 bp, synthetic construct
  misc_feature 1..20: note = primer
  source 1..20: mol_type = other DNA
tgctggtcgtgaccttactg

SEQ ID NO: 4 - DNA, 20 bp, synthetic construct
  misc_feature 1..20: note = primer
  source 1..20: mol_type = other DNA
cgaggtctccatctcttgct